European Patent Specification EP 3 924 473 B1, published January 28, 2026. Title: ENZYMATIC PRODUCTION OF MANNOSE. Applicant: BONUMOSE LLC. Application PCT/US20/17708. The sequence listing filed with the application follows.

SEQUENCE LISTING (2 sequences)

SEQ ID NO: 1 - protein, 223 aa, Thermobifida cellulosilytica TB100
MISDSDPQIPQAVLFDMDGTLIDTEPMWMDTEAEVAAAFGYTWTAEDQQRCLGGSAAAVADLIAERSGTRTPQSEIVAMLYAAVERRMAEGVPVRPGAKELLTELEAQGVPMALVTSTYRSLLTVALRAIGEHYFAVSVAGDEVTRNKPHPEPYLRAARLLGVDPRRCVAVEDSPTGVASAQAAGCTVVAVPHMASVPAAERRYVVGSLEEVDLAWLRRVSPA

SEQ ID NO: 2 - protein, 6 aa, Artificial Sequence
  motif
  misc_feature (3)..(5): Xaa can be any naturally occurring amino acid
GDXXXD